European Patent Application EP 4 116 313 A1, published January 11, 2023. Title: Cap analog for the 5'-end of eukaryotic messenger RNAs. Applicant: Westfälische Wilhelms-Universität Münster. The sequence listing filed with the application follows.

SEQUENCE LISTING (2 sequences)

SEQ ID NO: 1 - DNA, 27 bp, artificial
  forward primer
taatacgactcactatagggaaataag

SEQ ID NO: 2 - DNA, 21 bp, Artificial
  reverse primer
atccagtcgcgctgctctcgc